European Patent Specification EP 3 092 305 B1, published August 2, 2023. Title: Method of producing microglial cells. Applicant: KYUSHU UNIVERSITY NATIONAL UNIVERSITY CORPORATION. Application EP 15734968.9. The sequence listing filed with the application follows.

SEQUENCE LISTING (16 sequences)

SEQ ID NO: 1 - DNA, 23 bp, Artificial
  synthetic DNA
ttcaggaatcagaaaggacactc

SEQ ID NO: 2 - DNA, 20 bp, Artificial
  synthetic DNA
tctgcatttcagctcaggaa

SEQ ID NO: 3 - DNA, 27 bp, Artificial
  synthetic DNA
agtcaaagttattgttatgctgacaga

SEQ ID NO: 4 - DNA, 20 bp, Artificial
  synthetic DNA
tgctttccttctccccagta

SEQ ID NO: 5 - DNA, 21 bp, Artificial
  synthetic DNA
cagcctcttctccttcctgat

SEQ ID NO: 6 - DNA, 20 bp, Artificial
  synthetic DNA
gccagagggctgattagaga

SEQ ID NO: 7 - DNA, 19 bp, Artificial
  synthetic DNA
ggggaaaccaatgaaaagc

SEQ ID NO: 8 - DNA, 22 bp, Artificial
  synthetic DNA
acctcatcttgacacaggcata

SEQ ID NO: 9 - DNA, 18 bp, Artificial
  synthetic DNA
atggccctctgctcctgt

SEQ ID NO: 10 - DNA, 22 bp, Artificial
  synthetic DNA
aatctgccaggaggtatagacg

SEQ ID NO: 11 - DNA, 20 bp, Artificial
  synthetic DNA
tgggattcatttggttgttg

SEQ ID NO: 12 - DNA, 27 bp, Artificial
  synthetic DNA
caactggagtagattctgttttattca

SEQ ID NO: 13 - DNA, 20 bp, Artificial
  synthetic DNA
gagaccgagtcgccttatca

SEQ ID NO: 14 - DNA, 20 bp, Artificial
  synthetic DNA
ctgtgtgttgaggtcgctgt

SEQ ID NO: 15 - DNA, 20 bp, Artificial
  synthetic DNA
tctgagagcttcgaggatgc

SEQ ID NO: 16 - DNA, 20 bp, Artificial
  synthetic DNA
ggggatttctccttccaaga